European Patent Application EP 4 410 988 A1, published August 7, 2024. Title: An AAV2-vector variant for targeted transfer of genes. Applicant: UNIVERSITÄTSKLININUKUM HAMBURG-EPPENDORF. Application EP. The sequence listing filed with the application follows.

SEQUENCE LISTING (9 sequences)

SEQ ID NO: 1 - protein, 6 aa, synthetic construct
QVLXXR

SEQ ID NO: 2 - protein, 7 aa, synthetic construct
QVLXXRX

SEQ ID NO: 3 - protein, 7 aa, synthetic construct
QVLVYRE

SEQ ID NO: 4 - protein, 7 aa, synthetic construct
QVLDNRE

SEQ ID NO: 5 - protein, 7 aa, synthetic construct
QVLDYRA

SEQ ID NO: 6 - protein, 7 aa, synthetic construct
QVLVYLE

SEQ ID NO: 7 - protein, 7 aa, synthetic construct
QVLGYRK

SEQ ID NO: 8 - DNA, 19 bp, synthetic construct
  source 1..19: mol_type = other DNA
gggactttcctacttggca

SEQ ID NO: 9 - RNA, 19 nt, synthetic construct
  source 1..19: mol_type = other RNA
ggcggagttgttacgacat